European Patent Application EP 4 386 091 A1, published June 19, 2024. Title: A method for taxonomic classification up to species level of bacteria. Applicant: The BioArte Limited. The sequence listing filed with the application follows.

SEQUENCE LISTING (196 sequences)

SEQ ID NO: 1 - DNA, 42 bp, synthetic construct
  source 1..42: mol_type = other DNA
tttctgttggtgctgatattgcagrgttygatymtggctcag

SEQ ID NO: 2 - DNA, 42 bp, synthetic construct
  source 1..42: mol_type = other DNA
acttgcctgtcgctctatcttccggttaccttgttacgactt

SEQ ID NO: 3 - DNA, 19 bp, synthetic construct
  source 1..19: mol_type = other DNA
gtgccagcmgccgcggtaa

SEQ ID NO: 4 - DNA, 20 bp, synthetic construct
  source 1..20: mol_type = other DNA
ggactachvgggtwtctaat

SEQ ID NO: 5 - DNA, 59 bp, synthetic construct
  source 1..59: mol_type = other DNA
ggtgctgaagaaagttgtcggtgtctttgtgttaacctttctgttggtgctgatattgc

SEQ ID NO: 6 - DNA, 59 bp, synthetic construct
  source 1..59: mol_type = other DNA
ggtgctgtcgattccgtttgtagtcgtctgtttaacctttctgttggtgctgatattgc

SEQ ID NO: 7 - DNA, 59 bp, synthetic construct
  source 1..59: mol_type = other DNA
ggtgctggagtcttgtgtcccagttaccaggttaacctttctgttggtgctgatattgc

SEQ ID NO: 8 - DNA, 59 bp, synthetic construct
  source 1..59: mol_type = other DNA
ggtgctgttcggattctatcgtgtttccctattaacctttctgttggtgctgatattgc

SEQ ID NO: 9 - DNA, 59 bp, synthetic construct
  source 1..59: mol_type = other DNA
ggtgctgcttgtccagggtttgtgtaaccttttaacctttctgttggtgctgatattgc

SEQ ID NO: 10 - DNA, 59 bp, synthetic construct
  source 1..59: mol_type = other DNA
ggtgctgttctcgcaaaggcagaaagtagtcttaacctttctgttggtgctgatattgc

SEQ ID NO: 11 - DNA, 59 bp, synthetic construct
  source 1..59: mol_type = other DNA
ggtgctggtgttaccgtgggaatgaatccttttaacctttctgttggtgctgatattgc

SEQ ID NO: 12 - DNA, 59 bp, synthetic construct
  source 1..59: mol_type = other DNA
ggtgctgttcagggaacaaaccaagttacgtttaacctttctgttggtgctgatattgc

SEQ ID NO: 13 - DNA, 59 bp, synthetic construct
  source 1..59: mol_type = other DNA
ggtgctgaactaggcacagcgagtcttggttttaacctttctgttggtgctgatattgc

SEQ ID NO: 14 - DNA, 59 bp, synthetic construct
  source 1..59: mol_type = other DNA
ggtgctgaagcgttgaaacctttgtcctctcttaacctttctgttggtgctgatattgc

SEQ ID NO: 15 - DNA, 59 bp, synthetic construct
  source 1..59: mol_type = other DNA
ggtgctggtttcatctatcggagggaatggattaacctttctgttggtgctgatattgc

SEQ ID NO: 16 - DNA, 59 bp, synthetic construct
  source 1..59: mol_type = other DNA
ggtgctgcaggtagaaagaagcagaatcggattaacctttctgttggtgctgatattgc

SEQ ID NO: 17 - DNA, 59 bp, synthetic construct
  source 1..59: mol_type = other DNA
ggtgctgagaacgacttccatactcgtgtgattaacctttctgttggtgctgatattgc

SEQ ID NO: 18 - DNA, 59 bp, synthetic construct
  source 1..59: mol_type = other DNA
ggtgctgaacgagtctcttgggacccatagattaacctttctgttggtgctgatattgc

SEQ ID NO: 19 - DNA, 59 bp, synthetic construct
  source 1..59: mol_type = other DNA
ggtgctgaggtctacctcgctaacaccactgttaacctttctgttggtgctgatattgc

SEQ ID NO: 20 - DNA, 59 bp, synthetic construct
  source 1..59: mol_type = other DNA
ggtgctgcgtcaactgacagtggttcgtactttaacctttctgttggtgctgatattgc

SEQ ID NO: 21 - DNA, 59 bp, synthetic construct
  source 1..59: mol_type = other DNA
ggtgctgaccctccaggaaagtacctctgatttaacctttctgttggtgctgatattgc

SEQ ID NO: 22 - DNA, 59 bp, synthetic construct
  source 1..59: mol_type = other DNA
ggtgctgccaaacccaacaacctagataggcttaacctttctgttggtgctgatattgc

SEQ ID NO: 23 - DNA, 59 bp, synthetic construct
  source 1..59: mol_type = other DNA
ggtgctggttcctcgtgcagtgtcaagagatttaacctttctgttggtgctgatattgc

SEQ ID NO: 24 - DNA, 59 bp, synthetic construct
  source 1..59: mol_type = other DNA
ggtgctgttgcgtcctgttacgagaactcatttaacctttctgttggtgctgatattgc

SEQ ID NO: 25 - DNA, 59 bp, synthetic construct
  source 1..59: mol_type = other DNA
ggtgctggagcctctcattgtccgttctctattaacctttctgttggtgctgatattgc

SEQ ID NO: 26 - DNA, 59 bp, synthetic construct
  source 1..59: mol_type = other DNA
ggtgctgaccactgccatgtatcaaagtacgttaacctttctgttggtgctgatattgc

SEQ ID NO: 27 - DNA, 59 bp, synthetic construct
  source 1..59: mol_type = other DNA
ggtgctgcttactacccagtgaacctcctcgttaacctttctgttggtgctgatattgc

SEQ ID NO: 28 - DNA, 59 bp, synthetic construct
  source 1..59: mol_type = other DNA
ggtgctggcatagttctgcatgatgggttagttaacctttctgttggtgctgatattgc

SEQ ID NO: 29 - DNA, 59 bp, synthetic construct
  source 1..59: mol_type = other DNA
ggtgctggtaagttgggtatgcaacgcaatgttaacctttctgttggtgctgatattgc

SEQ ID NO: 30 - DNA, 59 bp, synthetic construct
  source 1..59: mol_type = other DNA
ggtgctgcatacagcgactacgcattctcatttaacctttctgttggtgctgatattgc

SEQ ID NO: 31 - DNA, 59 bp, synthetic construct
  source 1..59: mol_type = other DNA
ggtgctgcgacggttagattcacctcttacattaacctttctgttggtgctgatattgc

SEQ ID NO: 32 - DNA, 59 bp, synthetic construct
  source 1..59: mol_type = other DNA
ggtgctgtgaaacctaagaaggcaccgtatcttaacctttctgttggtgctgatattgc

SEQ ID NO: 33 - DNA, 59 bp, synthetic construct
  source 1..59: mol_type = other DNA
ggtgctgctagacaccttgggttgacagaccttaacctttctgttggtgctgatattgc

SEQ ID NO: 34 - DNA, 59 bp, synthetic construct
  source 1..59: mol_type = other DNA
ggtgctgtcagtgaggatctacttcgacccattaacctttctgttggtgctgatattgc

SEQ ID NO: 35 - DNA, 59 bp, synthetic construct
  source 1..59: mol_type = other DNA
ggtgctgtgcgtacagcaatcagttacattgttaacctttctgttggtgctgatattgc

SEQ ID NO: 36 - DNA, 59 bp, synthetic construct
  source 1..59: mol_type = other DNA
ggtgctgccagtagaagtccgacaacgtcatttaacctttctgttggtgctgatattgc

SEQ ID NO: 37 - DNA, 59 bp, synthetic construct
  source 1..59: mol_type = other DNA
ggtgctgcagacttggtacggttgggtaactttaacctttctgttggtgctgatattgc

SEQ ID NO: 38 - DNA, 59 bp, synthetic construct
  source 1..59: mol_type = other DNA
ggtgctgggacgaagaactcaagtcaaaggcttaacctttctgttggtgctgatattgc

SEQ ID NO: 39 - DNA, 59 bp, synthetic construct
  source 1..59: mol_type = other DNA
ggtgctgctacttacgaagctgagggactgcttaacctttctgttggtgctgatattgc

SEQ ID NO: 40 - DNA, 59 bp, synthetic construct
  source 1..59: mol_type = other DNA
ggtgctgatgtcccagttagaggaggaaacattaacctttctgttggtgctgatattgc

SEQ ID NO: 41 - DNA, 59 bp, synthetic construct
  source 1..59: mol_type = other DNA
ggtgctggcttgcgattgatgcttagtatcattaacctttctgttggtgctgatattgc

SEQ ID NO: 42 - DNA, 59 bp, synthetic construct
  source 1..59: mol_type = other DNA
ggtgctgaccacaggaggacgatacagagaattaacctttctgttggtgctgatattgc

SEQ ID NO: 43 - DNA, 59 bp, synthetic construct
  source 1..59: mol_type = other DNA
ggtgctgccacagtgtcaactagagcctctcttaacctttctgttggtgctgatattgc

SEQ ID NO: 44 - DNA, 59 bp, synthetic construct
  source 1..59: mol_type = other DNA
ggtgctgtagtttggatgaccaaggatagccttaacctttctgttggtgctgatattgc

SEQ ID NO: 45 - DNA, 59 bp, synthetic construct
  source 1..59: mol_type = other DNA
ggtgctgggagttcgtccagagaagtacacgttaacctttctgttggtgctgatattgc

SEQ ID NO: 46 - DNA, 59 bp, synthetic construct
  source 1..59: mol_type = other DNA
ggtgctgctacgtgtaaggcatacctgccagttaacctttctgttggtgctgatattgc

SEQ ID NO: 47 - DNA, 59 bp, synthetic construct
  source 1..59: mol_type = other DNA
ggtgctgctttcgttgttgactcgacggtagttaacctttctgttggtgctgatattgc

SEQ ID NO: 48 - DNA, 59 bp, synthetic construct
  source 1..59: mol_type = other DNA
ggtgctgagtagaaagggttccttcccactcttaacctttctgttggtgctgatattgc

SEQ ID NO: 49 - DNA, 59 bp, synthetic construct
  source 1..59: mol_type = other DNA
ggtgctggatccaacagagatgccttcagtgttaacctttctgttggtgctgatattgc

SEQ ID NO: 50 - DNA, 59 bp, synthetic construct
  source 1..59: mol_type = other DNA
ggtgctggctgtgttccacttcattctcctgttaacctttctgttggtgctgatattgc

SEQ ID NO: 51 - DNA, 59 bp, synthetic construct
  source 1..59: mol_type = other DNA
ggtgctggtgcaactttcccacaggtagttcttaacctttctgttggtgctgatattgc

SEQ ID NO: 52 - DNA, 59 bp, synthetic construct
  source 1..59: mol_type = other DNA
ggtgctgcatctggaacgtggtacacctgtattaacctttctgttggtgctgatattgc

SEQ ID NO: 53 - DNA, 59 bp, synthetic construct
  source 1..59: mol_type = other DNA
ggtgctgactggtgcagctttgaacatctagttaacctttctgttggtgctgatattgc

SEQ ID NO: 54 - DNA, 59 bp, synthetic construct
  source 1..59: mol_type = other DNA
ggtgctgatggactttggtaacttcctgcgtttaacctttctgttggtgctgatattgc

SEQ ID NO: 55 - DNA, 59 bp, synthetic construct
  source 1..59: mol_type = other DNA
ggtgctggttgaatgagcctactgggtcctcttaacctttctgttggtgctgatattgc

SEQ ID NO: 56 - DNA, 59 bp, synthetic construct
  source 1..59: mol_type = other DNA
ggtgctgtgagagacaagattgttcgtggacttaacctttctgttggtgctgatattgc

SEQ ID NO: 57 - DNA, 59 bp, synthetic construct
  source 1..59: mol_type = other DNA
ggtgctgagattcagaccgtctcatgcaaagttaacctttctgttggtgctgatattgc

SEQ ID NO: 58 - DNA, 59 bp, synthetic construct
  source 1..59: mol_type = other DNA
ggtgctgcaagagctttgactaaggagcatgttaacctttctgttggtgctgatattgc

SEQ ID NO: 59 - DNA, 59 bp, synthetic construct
  source 1..59: mol_type = other DNA
ggtgctgtggaagatgagaccctgatctacgttaacctttctgttggtgctgatattgc

SEQ ID NO: 60 - DNA, 59 bp, synthetic construct
  source 1..59: mol_type = other DNA
ggtgctgtcactactcaacaggtggcatgaattaacctttctgttggtgctgatattgc

SEQ ID NO: 61 - DNA, 59 bp, synthetic construct
  source 1..59: mol_type = other DNA
ggtgctggctaggtcaatctccttcggaagtttaacctttctgttggtgctgatattgc

SEQ ID NO: 62 - DNA, 59 bp, synthetic construct
  source 1..59: mol_type = other DNA
ggtgctgcaggttactcctccgtgagtctgattaacctttctgttggtgctgatattgc

SEQ ID NO: 63 - DNA, 59 bp, synthetic construct
  source 1..59: mol_type = other DNA
ggtgctgtcaatcaagaagggaaagcaaggtttaacctttctgttggtgctgatattgc

SEQ ID NO: 64 - DNA, 59 bp, synthetic construct
  source 1..59: mol_type = other DNA
ggtgctgcatgttcaaccaaggcttctatggttaacctttctgttggtgctgatattgc

SEQ ID NO: 65 - DNA, 59 bp, synthetic construct
  source 1..59: mol_type = other DNA
ggtgctgagagggtactatgtgcctcagcacttaacctttctgttggtgctgatattgc

SEQ ID NO: 66 - DNA, 59 bp, synthetic construct
  source 1..59: mol_type = other DNA
ggtgctgcacccacacttacttcaggacgtattaacctttctgttggtgctgatattgc

SEQ ID NO: 67 - DNA, 59 bp, synthetic construct
  source 1..59: mol_type = other DNA
ggtgctgttctgaagttcctgggtcttgaacttaacctttctgttggtgctgatattgc

SEQ ID NO: 68 - DNA, 59 bp, synthetic construct
  source 1..59: mol_type = other DNA
ggtgctggacagacaccgttcatcgactttcttaacctttctgttggtgctgatattgc

SEQ ID NO: 69 - DNA, 59 bp, synthetic construct
  source 1..59: mol_type = other DNA
ggtgctgttctcagtcttcctccagacaaggttaacctttctgttggtgctgatattgc

SEQ ID NO: 70 - DNA, 59 bp, synthetic construct
  source 1..59: mol_type = other DNA
ggtgctgccgatccttgtggcttctaacttcttaacctttctgttggtgctgatattgc

SEQ ID NO: 71 - DNA, 59 bp, synthetic construct
  source 1..59: mol_type = other DNA
ggtgctggtttgtcatactcgtgtgctcaccttaacctttctgttggtgctgatattgc

SEQ ID NO: 72 - DNA, 59 bp, synthetic construct
  source 1..59: mol_type = other DNA
ggtgctggaatctaagcaaacacgaaggtggttaacctttctgttggtgctgatattgc

SEQ ID NO: 73 - DNA, 59 bp, synthetic construct
  source 1..59: mol_type = other DNA
ggtgctgtacagtccgagcctcatgtgatctttaacctttctgttggtgctgatattgc

SEQ ID NO: 74 - DNA, 59 bp, synthetic construct
  source 1..59: mol_type = other DNA
ggtgctgaccgagatcctacgaatggagtgtttaacctttctgttggtgctgatattgc

SEQ ID NO: 75 - DNA, 59 bp, synthetic construct
  source 1..59: mol_type = other DNA
ggtgctgcctgggagcatcaggtagtaacagttaacctttctgttggtgctgatattgc

SEQ ID NO: 76 - DNA, 59 bp, synthetic construct
  source 1..59: mol_type = other DNA
ggtgctgtagctgactgtcttccataccgacttaacctttctgttggtgctgatattgc

SEQ ID NO: 77 - DNA, 59 bp, synthetic construct
  source 1..59: mol_type = other DNA
ggtgctgaagaaacaggatgacagaaccctcttaacctttctgttggtgctgatattgc

SEQ ID NO: 78 - DNA, 59 bp, synthetic construct
  source 1..59: mol_type = other DNA
ggtgctgtacaagcatcccaacacttccactttaacctttctgttggtgctgatattgc

SEQ ID NO: 79 - DNA, 59 bp, synthetic construct
  source 1..59: mol_type = other DNA
ggtgctggaccattgtgatgaaccctgttgtttaacctttctgttggtgctgatattgc

SEQ ID NO: 80 - DNA, 59 bp, synthetic construct
  source 1..59: mol_type = other DNA
ggtgctgatgcttgttacatcaaccctggacttaacctttctgttggtgctgatattgc

SEQ ID NO: 81 - DNA, 59 bp, synthetic construct
  source 1..59: mol_type = other DNA
ggtgctgcgacctgtttctcagggatacaacttaacctttctgttggtgctgatattgc

SEQ ID NO: 82 - DNA, 59 bp, synthetic construct
  source 1..59: mol_type = other DNA
ggtgctgaacaaccgaacctttgaatcagaattaacctttctgttggtgctgatattgc

SEQ ID NO: 83 - DNA, 59 bp, synthetic construct
  source 1..59: mol_type = other DNA
ggtgctgtctcggagatagttctcactgctgttaacctttctgttggtgctgatattgc

SEQ ID NO: 84 - DNA, 59 bp, synthetic construct
  source 1..59: mol_type = other DNA
ggtgctgcggatgaacataggatagcgattcttaacctttctgttggtgctgatattgc

SEQ ID NO: 85 - DNA, 59 bp, synthetic construct
  source 1..59: mol_type = other DNA
ggtgctgcctcatcttgtgaagttgtttcggttaacctttctgttggtgctgatattgc

SEQ ID NO: 86 - DNA, 59 bp, synthetic construct
  source 1..59: mol_type = other DNA
ggtgctgacggtatgtcgagttccaggactattaacctttctgttggtgctgatattgc

SEQ ID NO: 87 - DNA, 59 bp, synthetic construct
  source 1..59: mol_type = other DNA
ggtgctgtggcttgatctaggtaaggtcgaattaacctttctgttggtgctgatattgc

SEQ ID NO: 88 - DNA, 59 bp, synthetic construct
  source 1..59: mol_type = other DNA
ggtgctggtagtggacctagaacctgtgccattaacctttctgttggtgctgatattgc

SEQ ID NO: 89 - DNA, 59 bp, synthetic construct
  source 1..59: mol_type = other DNA
ggtgctgaacggaggagttagttggatgatcttaacctttctgttggtgctgatattgc

SEQ ID NO: 90 - DNA, 59 bp, synthetic construct
  source 1..59: mol_type = other DNA
ggtgctgaggtgatcccaacaagcgtaagtattaacctttctgttggtgctgatattgc

SEQ ID NO: 91 - DNA, 59 bp, synthetic construct
  source 1..59: mol_type = other DNA
ggtgctgtacatgctcctgttgttagggaggttaacctttctgttggtgctgatattgc

SEQ ID NO: 92 - DNA, 59 bp, synthetic construct
  source 1..59: mol_type = other DNA
ggtgctgtcttctactaccgatccgaagcagttaacctttctgttggtgctgatattgc

SEQ ID NO: 93 - DNA, 59 bp, synthetic construct
  source 1..59: mol_type = other DNA
ggtgctgacagcatcaatgtttggctagttgttaacctttctgttggtgctgatattgc

SEQ ID NO: 94 - DNA, 59 bp, synthetic construct
  source 1..59: mol_type = other DNA
ggtgctggatgtagagggtacggtttgaggcttaacctttctgttggtgctgatattgc

SEQ ID NO: 95 - DNA, 59 bp, synthetic construct
  source 1..59: mol_type = other DNA
ggtgctgggctccataggaactcacgctactttaacctttctgttggtgctgatattgc

SEQ ID NO: 96 - DNA, 59 bp, synthetic construct
  source 1..59: mol_type = other DNA
ggtgctgttgtgagtggaaagatacaggaccttaacctttctgttggtgctgatattgc

SEQ ID NO: 97 - DNA, 59 bp, synthetic construct
  source 1..59: mol_type = other DNA
ggtgctgagtttccatcacttcagacttgggttaacctttctgttggtgctgatattgc

SEQ ID NO: 98 - DNA, 59 bp, synthetic construct
  source 1..59: mol_type = other DNA
ggtgctggattgtcctcaaactgccacctacttaacctttctgttggtgctgatattgc

SEQ ID NO: 99 - DNA, 59 bp, synthetic construct
  source 1..59: mol_type = other DNA
ggtgctgcctgtctggaagaagaatggacttttaacctttctgttggtgctgatattgc

SEQ ID NO: 100 - DNA, 59 bp, synthetic construct
  source 1..59: mol_type = other DNA
ggtgctgctgaacggtcatagagtccaccatttaacctttctgttggtgctgatattgc

SEQ ID NO: 101 - DNA, 60 bp, synthetic construct
  source 1..60: mol_type = other DNA
ggtgctgaagaaagttgtcggtgtctttgtgttaacctacttgcctgtcgctctatcttc

SEQ ID NO: 102 - DNA, 60 bp, synthetic construct
  source 1..60: mol_type = other DNA
ggtgctgtcgattccgtttgtagtcgtctgtttaacctacttgcctgtcgctctatcttc

SEQ ID NO: 103 - DNA, 60 bp, synthetic construct
  source 1..60: mol_type = other DNA
ggtgctggagtcttgtgtcccagttaccaggttaacctacttgcctgtcgctctatcttc

SEQ ID NO: 104 - DNA, 60 bp, synthetic construct
  source 1..60: mol_type = other DNA
ggtgctgttcggattctatcgtgtttccctattaacctacttgcctgtcgctctatcttc

SEQ ID NO: 105 - DNA, 60 bp, synthetic construct
  source 1..60: mol_type = other DNA
ggtgctgcttgtccagggtttgtgtaaccttttaacctacttgcctgtcgctctatcttc

SEQ ID NO: 106 - DNA, 60 bp, synthetic construct
  source 1..60: mol_type = other DNA
ggtgctgttctcgcaaaggcagaaagtagtcttaacctacttgcctgtcgctctatcttc

SEQ ID NO: 107 - DNA, 60 bp, synthetic construct
  source 1..60: mol_type = other DNA
ggtgctggtgttaccgtgggaatgaatccttttaacctacttgcctgtcgctctatcttc

SEQ ID NO: 108 - DNA, 60 bp, synthetic construct
  source 1..60: mol_type = other DNA
ggtgctgttcagggaacaaaccaagttacgtttaacctacttgcctgtcgctctatcttc

SEQ ID NO: 109 - DNA, 60 bp, synthetic construct
  source 1..60: mol_type = other DNA
ggtgctgaactaggcacagcgagtcttggttttaacctacttgcctgtcgctctatcttc

SEQ ID NO: 110 - DNA, 60 bp, synthetic construct
  source 1..60: mol_type = other DNA
ggtgctgaagcgttgaaacctttgtcctctcttaacctacttgcctgtcgctctatcttc

SEQ ID NO: 111 - DNA, 60 bp, synthetic construct
  source 1..60: mol_type = other DNA
ggtgctggtttcatctatcggagggaatggattaacctacttgcctgtcgctctatcttc

SEQ ID NO: 112 - DNA, 60 bp, synthetic construct
  source 1..60: mol_type = other DNA
ggtgctgcaggtagaaagaagcagaatcggattaacctacttgcctgtcgctctatcttc

SEQ ID NO: 113 - DNA, 60 bp, synthetic construct
  source 1..60: mol_type = other DNA
ggtgctgagaacgacttccatactcgtgtgattaacctacttgcctgtcgctctatcttc

SEQ ID NO: 114 - DNA, 60 bp, synthetic construct
  source 1..60: mol_type = other DNA
ggtgctgaacgagtctcttgggacccatagattaacctacttgcctgtcgctctatcttc

SEQ ID NO: 115 - DNA, 60 bp, synthetic construct
  source 1..60: mol_type = other DNA
ggtgctgaggtctacctcgctaacaccactgttaacctacttgcctgtcgctctatcttc

SEQ ID NO: 116 - DNA, 60 bp, synthetic construct
  source 1..60: mol_type = other DNA
ggtgctgcgtcaactgacagtggttcgtactttaacctacttgcctgtcgctctatcttc

SEQ ID NO: 117 - DNA, 60 bp, synthetic construct
  source 1..60: mol_type = other DNA
ggtgctgaccctccaggaaagtacctctgatttaacctacttgcctgtcgctctatcttc

SEQ ID NO: 118 - DNA, 60 bp, synthetic construct
  source 1..60: mol_type = other DNA
ggtgctgccaaacccaacaacctagataggcttaacctacttgcctgtcgctctatcttc

SEQ ID NO: 119 - DNA, 60 bp, synthetic construct
  source 1..60: mol_type = other DNA
ggtgctggttcctcgtgcagtgtcaagagatttaacctacttgcctgtcgctctatcttc

SEQ ID NO: 120 - DNA, 60 bp, synthetic construct
  source 1..60: mol_type = other DNA
ggtgctgttgcgtcctgttacgagaactcatttaacctacttgcctgtcgctctatcttc

SEQ ID NO: 121 - DNA, 60 bp, synthetic construct
  source 1..60: mol_type = other DNA
ggtgctggagcctctcattgtccgttctctattaacctacttgcctgtcgctctatcttc

SEQ ID NO: 122 - DNA, 60 bp, synthetic construct
  source 1..60: mol_type = other DNA
ggtgctgaccactgccatgtatcaaagtacgttaacctacttgcctgtcgctctatcttc

SEQ ID NO: 123 - DNA, 60 bp, synthetic construct
  source 1..60: mol_type = other DNA
ggtgctgcttactacccagtgaacctcctcgttaacctacttgcctgtcgctctatcttc

SEQ ID NO: 124 - DNA, 60 bp, synthetic construct
  source 1..60: mol_type = other DNA
ggtgctggcatagttctgcatgatgggttagttaacctacttgcctgtcgctctatcttc

SEQ ID NO: 125 - DNA, 60 bp, synthetic construct
  source 1..60: mol_type = other DNA
ggtgctggtaagttgggtatgcaacgcaatgttaacctacttgcctgtcgctctatcttc

SEQ ID NO: 126 - DNA, 60 bp, synthetic construct
  source 1..60: mol_type = other DNA
ggtgctgcatacagcgactacgcattctcatttaacctacttgcctgtcgctctatcttc

SEQ ID NO: 127 - DNA, 60 bp, synthetic construct
  source 1..60: mol_type = other DNA
ggtgctgcgacggttagattcacctcttacattaacctacttgcctgtcgctctatcttc

SEQ ID NO: 128 - DNA, 60 bp, synthetic construct
  source 1..60: mol_type = other DNA
ggtgctgtgaaacctaagaaggcaccgtatcttaacctacttgcctgtcgctctatcttc

SEQ ID NO: 129 - DNA, 60 bp, synthetic construct
  source 1..60: mol_type = other DNA
ggtgctgctagacaccttgggttgacagaccttaacctacttgcctgtcgctctatcttc

SEQ ID NO: 130 - DNA, 60 bp, synthetic construct
  source 1..60: mol_type = other DNA
ggtgctgtcagtgaggatctacttcgacccattaacctacttgcctgtcgctctatcttc

SEQ ID NO: 131 - DNA, 60 bp, synthetic construct
  source 1..60: mol_type = other DNA
ggtgctgtgcgtacagcaatcagttacattgttaacctacttgcctgtcgctctatcttc

SEQ ID NO: 132 - DNA, 60 bp, synthetic construct
  source 1..60: mol_type = other DNA
ggtgctgccagtagaagtccgacaacgtcatttaacctacttgcctgtcgctctatcttc

SEQ ID NO: 133 - DNA, 60 bp, synthetic construct
  source 1..60: mol_type = other DNA
ggtgctgcagacttggtacggttgggtaactttaacctacttgcctgtcgctctatcttc

SEQ ID NO: 134 - DNA, 60 bp, synthetic construct
  source 1..60: mol_type = other DNA
ggtgctgggacgaagaactcaagtcaaaggcttaacctacttgcctgtcgctctatcttc

SEQ ID NO: 135 - DNA, 60 bp, synthetic construct
  source 1..60: mol_type = other DNA
ggtgctgctacttacgaagctgagggactgcttaacctacttgcctgtcgctctatcttc

SEQ ID NO: 136 - DNA, 60 bp, synthetic construct
  source 1..60: mol_type = other DNA
ggtgctgatgtcccagttagaggaggaaacattaacctacttgcctgtcgctctatcttc

SEQ ID NO: 137 - DNA, 60 bp, synthetic construct
  source 1..60: mol_type = other DNA
ggtgctggcttgcgattgatgcttagtatcattaacctacttgcctgtcgctctatcttc

SEQ ID NO: 138 - DNA, 60 bp, synthetic construct
  source 1..60: mol_type = other DNA
ggtgctgaccacaggaggacgatacagagaattaacctacttgcctgtcgctctatcttc

SEQ ID NO: 139 - DNA, 60 bp, synthetic construct
  source 1..60: mol_type = other DNA
ggtgctgccacagtgtcaactagagcctctcttaacctacttgcctgtcgctctatcttc

SEQ ID NO: 140 - DNA, 60 bp, synthetic construct
  source 1..60: mol_type = other DNA
ggtgctgtagtttggatgaccaaggatagccttaacctacttgcctgtcgctctatcttc

SEQ ID NO: 141 - DNA, 60 bp, synthetic construct
  source 1..60: mol_type = other DNA
ggtgctgggagttcgtccagagaagtacacgttaacctacttgcctgtcgctctatcttc

SEQ ID NO: 142 - DNA, 60 bp, synthetic construct
  source 1..60: mol_type = other DNA
ggtgctgctacgtgtaaggcatacctgccagttaacctacttgcctgtcgctctatcttc

SEQ ID NO: 143 - DNA, 60 bp, synthetic construct
  source 1..60: mol_type = other DNA
ggtgctgctttcgttgttgactcgacggtagttaacctacttgcctgtcgctctatcttc

SEQ ID NO: 144 - DNA, 60 bp, synthetic construct
  source 1..60: mol_type = other DNA
ggtgctgagtagaaagggttccttcccactcttaacctacttgcctgtcgctctatcttc

SEQ ID NO: 145 - DNA, 60 bp, synthetic construct
  source 1..60: mol_type = other DNA
ggtgctggatccaacagagatgccttcagtgttaacctacttgcctgtcgctctatcttc

SEQ ID NO: 146 - DNA, 60 bp, synthetic construct
  source 1..60: mol_type = other DNA
ggtgctggctgtgttccacttcattctcctgttaacctacttgcctgtcgctctatcttc

SEQ ID NO: 147 - DNA, 60 bp, synthetic construct
  source 1..60: mol_type = other DNA
ggtgctggtgcaactttcccacaggtagttcttaacctacttgcctgtcgctctatcttc

SEQ ID NO: 148 - DNA, 60 bp, synthetic construct
  source 1..60: mol_type = other DNA
ggtgctgcatctggaacgtggtacacctgtattaacctacttgcctgtcgctctatcttc

SEQ ID NO: 149 - DNA, 60 bp, synthetic construct
  source 1..60: mol_type = other DNA
ggtgctgactggtgcagctttgaacatctagttaacctacttgcctgtcgctctatcttc

SEQ ID NO: 150 - DNA, 60 bp, synthetic construct
  source 1..60: mol_type = other DNA
ggtgctgatggactttggtaacttcctgcgtttaacctacttgcctgtcgctctatcttc

SEQ ID NO: 151 - DNA, 60 bp, synthetic construct
  source 1..60: mol_type = other DNA
ggtgctggttgaatgagcctactgggtcctcttaacctacttgcctgtcgctctatcttc

SEQ ID NO: 152 - DNA, 60 bp, synthetic construct
  source 1..60: mol_type = other DNA
ggtgctgtgagagacaagattgttcgtggacttaacctacttgcctgtcgctctatcttc

SEQ ID NO: 153 - DNA, 60 bp, synthetic construct
  source 1..60: mol_type = other DNA
ggtgctgagattcagaccgtctcatgcaaagttaacctacttgcctgtcgctctatcttc

SEQ ID NO: 154 - DNA, 60 bp, synthetic construct
  source 1..60: mol_type = other DNA
ggtgctgcaagagctttgactaaggagcatgttaacctacttgcctgtcgctctatcttc

SEQ ID NO: 155 - DNA, 60 bp, synthetic construct
  source 1..60: mol_type = other DNA
ggtgctgtggaagatgagaccctgatctacgttaacctacttgcctgtcgctctatcttc

SEQ ID NO: 156 - DNA, 60 bp, synthetic construct
  source 1..60: mol_type = other DNA
ggtgctgtcactactcaacaggtggcatgaattaacctacttgcctgtcgctctatcttc

SEQ ID NO: 157 - DNA, 60 bp, synthetic construct
  source 1..60: mol_type = other DNA
ggtgctggctaggtcaatctccttcggaagtttaacctacttgcctgtcgctctatcttc

SEQ ID NO: 158 - DNA, 60 bp, synthetic construct
  source 1..60: mol_type = other DNA
ggtgctgcaggttactcctccgtgagtctgattaacctacttgcctgtcgctctatcttc

SEQ ID NO: 159 - DNA, 60 bp, synthetic construct
  source 1..60: mol_type = other DNA
ggtgctgtcaatcaagaagggaaagcaaggtttaacctacttgcctgtcgctctatcttc

SEQ ID NO: 160 - DNA, 60 bp, synthetic construct
  source 1..60: mol_type = other DNA
ggtgctgcatgttcaaccaaggcttctatggttaacctacttgcctgtcgctctatcttc

SEQ ID NO: 161 - DNA, 60 bp, synthetic construct
  source 1..60: mol_type = other DNA
ggtgctgagagggtactatgtgcctcagcacttaacctacttgcctgtcgctctatcttc

SEQ ID NO: 162 - DNA, 60 bp, synthetic construct
  source 1..60: mol_type = other DNA
ggtgctgcacccacacttacttcaggacgtattaacctacttgcctgtcgctctatcttc

SEQ ID NO: 163 - DNA, 60 bp, synthetic construct
  source 1..60: mol_type = other DNA
ggtgctgttctgaagttcctgggtcttgaacttaacctacttgcctgtcgctctatcttc

SEQ ID NO: 164 - DNA, 60 bp, synthetic construct
  source 1..60: mol_type = other DNA
ggtgctggacagacaccgttcatcgactttcttaacctacttgcctgtcgctctatcttc

SEQ ID NO: 165 - DNA, 60 bp, synthetic construct
  source 1..60: mol_type = other DNA
ggtgctgttctcagtcttcctccagacaaggttaacctacttgcctgtcgctctatcttc

SEQ ID NO: 166 - DNA, 60 bp, synthetic construct
  source 1..60: mol_type = other DNA
ggtgctgccgatccttgtggcttctaacttcttaacctacttgcctgtcgctctatcttc

SEQ ID NO: 167 - DNA, 60 bp, synthetic construct
  source 1..60: mol_type = other DNA
ggtgctggtttgtcatactcgtgtgctcaccttaacctacttgcctgtcgctctatcttc

SEQ ID NO: 168 - DNA, 60 bp, synthetic construct
  source 1..60: mol_type = other DNA
ggtgctggaatctaagcaaacacgaaggtggttaacctacttgcctgtcgctctatcttc

SEQ ID NO: 169 - DNA, 60 bp, synthetic construct
  source 1..60: mol_type = other DNA
ggtgctgtacagtccgagcctcatgtgatctttaacctacttgcctgtcgctctatcttc

SEQ ID NO: 170 - DNA, 60 bp, synthetic construct
  source 1..60: mol_type = other DNA
ggtgctgaccgagatcctacgaatggagtgtttaacctacttgcctgtcgctctatcttc

SEQ ID NO: 171 - DNA, 60 bp, synthetic construct
  source 1..60: mol_type = other DNA
ggtgctgcctgggagcatcaggtagtaacagttaacctacttgcctgtcgctctatcttc

SEQ ID NO: 172 - DNA, 60 bp, synthetic construct
  source 1..60: mol_type = other DNA
ggtgctgtagctgactgtcttccataccgacttaacctacttgcctgtcgctctatcttc

SEQ ID NO: 173 - DNA, 60 bp, synthetic construct
  source 1..60: mol_type = other DNA
ggtgctgaagaaacaggatgacagaaccctcttaacctacttgcctgtcgctctatcttc

SEQ ID NO: 174 - DNA, 60 bp, synthetic construct
  source 1..60: mol_type = other DNA
ggtgctgtacaagcatcccaacacttccactttaacctacttgcctgtcgctctatcttc

SEQ ID NO: 175 - DNA, 60 bp, synthetic construct
  source 1..60: mol_type = other DNA
ggtgctggaccattgtgatgaaccctgttgtttaacctacttgcctgtcgctctatcttc

SEQ ID NO: 176 - DNA, 60 bp, synthetic construct
  source 1..60: mol_type = other DNA
ggtgctgatgcttgttacatcaaccctggacttaacctacttgcctgtcgctctatcttc

SEQ ID NO: 177 - DNA, 60 bp, synthetic construct
  source 1..60: mol_type = other DNA
ggtgctgcgacctgtttctcagggatacaacttaacctacttgcctgtcgctctatcttc

SEQ ID NO: 178 - DNA, 60 bp, synthetic construct
  source 1..60: mol_type = other DNA
ggtgctgaacaaccgaacctttgaatcagaattaacctacttgcctgtcgctctatcttc

SEQ ID NO: 179 - DNA, 60 bp, synthetic construct
  source 1..60: mol_type = other DNA
ggtgctgtctcggagatagttctcactgctgttaacctacttgcctgtcgctctatcttc

SEQ ID NO: 180 - DNA, 60 bp, synthetic construct
  source 1..60: mol_type = other DNA
ggtgctgcggatgaacataggatagcgattcttaacctacttgcctgtcgctctatcttc

SEQ ID NO: 181 - DNA, 60 bp, synthetic construct
  source 1..60: mol_type = other DNA
ggtgctgcctcatcttgtgaagttgtttcggttaacctacttgcctgtcgctctatcttc

SEQ ID NO: 182 - DNA, 60 bp, synthetic construct
  source 1..60: mol_type = other DNA
ggtgctgacggtatgtcgagttccaggactattaacctacttgcctgtcgctctatcttc

SEQ ID NO: 183 - DNA, 60 bp, synthetic construct
  source 1..60: mol_type = other DNA
ggtgctgtggcttgatctaggtaaggtcgaattaacctacttgcctgtcgctctatcttc

SEQ ID NO: 184 - DNA, 60 bp, synthetic construct
  source 1..60: mol_type = other DNA
ggtgctggtagtggacctagaacctgtgccattaacctacttgcctgtcgctctatcttc

SEQ ID NO: 185 - DNA, 60 bp, synthetic construct
  source 1..60: mol_type = other DNA
ggtgctgaacggaggagttagttggatgatcttaacctacttgcctgtcgctctatcttc

SEQ ID NO: 186 - DNA, 60 bp, synthetic construct
  source 1..60: mol_type = other DNA
ggtgctgaggtgatcccaacaagcgtaagtattaacctacttgcctgtcgctctatcttc

SEQ ID NO: 187 - DNA, 60 bp, synthetic construct
  source 1..60: mol_type = other DNA
ggtgctgtacatgctcctgttgttagggaggttaacctacttgcctgtcgctctatcttc

SEQ ID NO: 188 - DNA, 60 bp, synthetic construct
  source 1..60: mol_type = other DNA
ggtgctgtcttctactaccgatccgaagcagttaacctacttgcctgtcgctctatcttc

SEQ ID NO: 189 - DNA, 60 bp, synthetic construct
  source 1..60: mol_type = other DNA
ggtgctgacagcatcaatgtttggctagttgttaacctacttgcctgtcgctctatcttc

SEQ ID NO: 190 - DNA, 60 bp, synthetic construct
  source 1..60: mol_type = other DNA
ggtgctggatgtagagggtacggtttgaggcttaacctacttgcctgtcgctctatcttc

SEQ ID NO: 191 - DNA, 60 bp, synthetic construct
  source 1..60: mol_type = other DNA
ggtgctgggctccataggaactcacgctactttaacctacttgcctgtcgctctatcttc

SEQ ID NO: 192 - DNA, 60 bp, synthetic construct
  source 1..60: mol_type = other DNA
ggtgctgttgtgagtggaaagatacaggaccttaacctacttgcctgtcgctctatcttc

SEQ ID NO: 193 - DNA, 60 bp, synthetic construct
  source 1..60: mol_type = other DNA
ggtgctgagtttccatcacttcagacttgggttaacctacttgcctgtcgctctatcttc

SEQ ID NO: 194 - DNA, 60 bp, synthetic construct
  source 1..60: mol_type = other DNA
ggtgctggattgtcctcaaactgccacctacttaacctacttgcctgtcgctctatcttc

SEQ ID NO: 195 - DNA, 60 bp, synthetic construct
  source 1..60: mol_type = other DNA
ggtgctgcctgtctggaagaagaatggacttttaacctacttgcctgtcgctctatcttc

SEQ ID NO: 196 - DNA, 60 bp, synthetic construct
  source 1..60: mol_type = other DNA
ggtgctgctgaacggtcatagagtccaccatttaacctacttgcctgtcgctctatcttc